European Patent Application EP 4 810 112 A2, published September 23, 2026. Title: NOVEL METHODS OF ADMINISTERING FVIII MIMETICS. Applicant: NOVO NORDISK A/S. The sequence listing filed with the application follows.

SEQUENCE LISTING (22 sequences)

SEQ ID NO: 1 - protein, 415 aa, Homo sapiens
YNSGKLEEFVQGNLERECMEEKCSFEEAREVFENTERTTEFWKQYVDGDQCESNPCLNGGSCKDDINSYECWCPFGFEGKNCELDVTCNIKNGRCEQFCKNSADNKVVCSCTEGYRLAENQKSCEPAVPFPCGRVSVSQTSKLTRAEAVFPDVDYVNSTEAETILDNITQSTQSFNDFTRVVGGEDAKPGQFPWQVVLNGKVDAFCGGSIVNEKWIVTAAHCVETGVKITVVAGEHNIEETEHTEQKRNVIRIIPHHNYNAAINKYNHDIALLELDEPLVLNSYVTPICIADKEYTNIFLKFGSGYVSGWGRVFHKGRSALVLQYLRVPLVDRATCLRSTKFTIYNNMFCAGFHEGGRDSCQGDSGGPHVTEVEGTSFLTGIISWGEECAMKGKYGIYTKVSRYVNWIKEKTKLT

SEQ ID NO: 2 - protein, 448 aa, Homo sapiens [sequence omitted]

SEQ ID NO: 3 - protein, 5 aa, synthetic construct
  REGION 1..5: note = HCDR1
DYAMH

SEQ ID NO: 4 - protein, 17 aa, synthetic construct
  REGION 1..17: note = HCDR2
GISWRGDIGGYVKSVKG

SEQ ID NO: 5 - protein, 13 aa, synthetic construct
  REGION 1..13: note = HCDR3
SYGSGSFYNAFDS

SEQ ID NO: 6 - protein, 122 aa, synthetic construct
  REGION 1..122: note = Artificial
EVQLVESGGGLVQPGRSLRLSCAASGFTFHDYAMHWVRQVPGKGLEWVSGISWRGDIGGYVKSVKGRFTISRDNAKNSLYLQMNSLRAEDTALYYCVKSYGSGSFYNAFDSWGQGTLVTVSS

SEQ ID NO: 7 - protein, 448 aa, synthetic construct
  REGION 1..448: note = Artificial, anti-FIX heavy chain
EVQLVESGGGLVQPGRSLRLSCAASGFTFHDYAMHWVRQVPGKGLEWVSGISWRGDIGGYVKSVKGRFTISRDNAKNSLYLQMNSLRAEDTALYYCVKSYGSGSFYNAFDSWGQGTLVTVSSASTKGPSVFPLAPCSRSTSESTAALGCLVKDYFPEPVTVSWNSGALTSGVHTFPAVLQSSGLYSLSSVVTVPSSSLGTKTYTCNVDHKPSNTKVDKRVESKYGPPCPPCPAPEFLGGPSVFLFPPKPKDTLMISRTPEVTCVVVDVSQEDPEVQFNWYVDGVEVHNAKTKPREEQFNSTYRVVSVLTVLHQDWLNGKEYKCKVSNKGLPSSIEKTISKAKGQPREPQVYTLPPSQEEMTKNQVSLTCLVKGFYPSDIAVEWESNGQPENNYKTTPPVLDSDGSFFLYSRLTVDKSRWQEGNVFSCSVMHEALHNHYTQKSLSLSLG

SEQ ID NO: 8 - protein, 11 aa, synthetic construct
  REGION 1..11: note = LCDR1
RASQSISSWLA

SEQ ID NO: 9 - protein, 7 aa, synthetic construct
  REGION 1..7: note = LCDR2
KASKLER

SEQ ID NO: 10 - protein, 9 aa, synthetic construct
  REGION 1..9: note = LCDR3
LEYSSYIRT

SEQ ID NO: 11 - protein, 107 aa, synthetic construct
  REGION 1..107: note = anti-FIX(a) VL
DIQMTQSPSTLSASVGDRVTITCRASQSISSWLAWYQQKPGKAPKFLIYKASKLERGTPSRFSGSGSGTEFSLTISSLQPDDFATYYCLEYSSYIRTFGQGTKVEIK

SEQ ID NO: 12 - protein, 214 aa, synthetic construct
  REGION 1..214: note = anti-FIX light chain
DIQMTQSPSTLSASVGDRVTITCRASQSISSWLAWYQQKPGKAPKFLIYKASKLERGTPSRFSGSGSGTEFSLTISSLQPDDFATYYCLEYSSYIRTFGQGTKVEIKRTVAAPSVFIFPPSDEQLKSGTASVVCLLNNFYPREAKVQWKVDNALQSGNSQESVTEQDSKDSTYSLSSTLTLSKADYEKHKVYACEVTHQGLSSPVTKSFNRGEC

SEQ ID NO: 13 - protein, 5 aa, synthetic construct
  REGION 1..5: note = anti-FX(a) HCDR1
TSWIV

SEQ ID NO: 14 - protein, 17 aa, synthetic construct
  REGION 1..17: note = anti-FX(a) HCDR2
MIDPSDSFTSYSPSFQG

SEQ ID NO: 15 - protein, 11 aa, synthetic construct
  REGION 1..11: note = anti-FX(a) HCDR3
LHYYNSEEFDV

SEQ ID NO: 16 - protein, 120 aa, synthetic construct
  REGION 1..120: note = anti-FX(a) VH
EVQLVQSGAEVKKPGESLRISCKGSGYSFSTSWIVWVRQMPGKGLEWMGMIDPSDSFTSYSPSFQGHVTISADKSISTAYLQWSSLKASDTAMYYCARLHYYNSEEFDVWGQGTLVTVSS

SEQ ID NO: 17 - protein, 446 aa, synthetic construct
  REGION 1..446: note = Artificial, anti-FX heavy chain
EVQLVQSGAEVKKPGESLRISCKGSGYSFSTSWIVWVRQMPGKGLEWMGMIDPSDSFTSYSPSFQGHVTISADKSISTAYLQWSSLKASDTAMYYCARLHYYNSEEFDVWGQGTLVTVSSASTKGPSVFPLAPCSRSTSESTAALGCLVKDYFPEPVTVSWNSGALTSGVHTFPAVLQSSGLYSLSSVVTVPSSSLGTKTYTCNVDHKPSNTKVDKRVESKYGPPCPPCPAPEFLGGPSVFLFPPKPKDTLMISRTPEVTCVVVDVSQEDPEVQFNWYVDGVEVHNAKTKPREEQFNSTYRVVSVLTVLHQDWLNGKEYKCKVSNKGLPSSIEKTISKAKGQPREPQVYTLPPSQEEMTKNQVSLTCLVKGFYPSDIAVEWESNGQPENNYKTTPPVLDSDGSFLLYSKLTVDKSRWQEGNVFSCSVMHEALHNHYTQKSLSLSLG

SEQ ID NO: 18 - protein, 12 aa, synthetic construct
  REGION 1..12: note = anti-FX(a) LCDR1
RASQSVSSSYLA

SEQ ID NO: 19 - protein, 7 aa, synthetic construct
  REGION 1..7: note = anti-FX(a) LCDR2
GQSSRTR

SEQ ID NO: 20 - protein, 10 aa, synthetic construct
  REGION 1..10: note = anti-FX(a) LCDR3
QQFGDSQLFT

SEQ ID NO: 21 - protein, 109 aa, synthetic construct
  REGION 1..109: note = anti-FX(a) VL
EIVLTQSPGTLSLSPGERATLSCRASQSVSSSYLAWYQQKPGQAPRLLIYGQSSRTRGIPDRFSGSGSGTDFTLTISRLEPEDFAVYYCQQFGDSQLFTFGQGTKLEIK

SEQ ID NO: 22 - protein, 216 aa, synthetic construct
  REGION 1..216: note = Artificial, anti-FX light chain
EIVLTQSPGTLSLSPGERATLSCRASQSVSSSYLAWYQQKPGQAPRLLIYGQSSRTRGIPDRFSGSGSGTDFTLTISRLEPEDFAVYYCQQFGDSQLFTFGQGTKLEIKRTVAAPSVFIFPPSDEQLKSGTASVVCLLNNFYPREAKVQWKVDNALQSGNSQESVTEQDSKDSTYSLSSTLTLSKADYEKHKVYACEVTHQGLSSPVTKSFNRGEC